European Patent Application EP 4 556 570 A1, published May 21, 2025. Title: Improved production of bacterial cellulose. Applicant: ETH Zurich. The sequence listing filed with the application follows.

SEQUENCE LISTING (13 sequences)

SEQ ID NO: 1 - DNA, 2264 bp, Komagataeibacter sucrofermentans
  source 1..2264: mol_type = genomic DNA
cacgaggccgcacggctgatctttccttcttgtgtctgtccactgtggatggttgtgggctccctgcgctcaaccggtagtgcaagtggtttcttttttggacgactattggccattattttgccttttttgcggaacagcgccttaatgctgagcagcaggctccacaggctgcgtagcggtctgtcatcctcataattgttccattgcagccaggcatcagcccgcccgaacacgaagcggacaatatcgcgttccgtatcaaggtcattattgtcccatgtgaacacggccttgccattcgtgcagcgcagcatggtggcgggaatatcgatttcctcgccatcaagcacggcatggatacgtttcttgacaggccccgtggtgacatcgggcaaggggatgtgcacggcaacaccacccatggaaacatcctgggtcatgccgtgcgtcgcattataataggtatggggctgcccttcggcaggcgcatcgtaaaccgttaccgggatatgcgcttcgacacgatggttgtaacggacctgcttggtctcgcgccccacggcaatggcagcgaaaaggatgatgagactgatcagcgcccaggcgcagttcaggagataagcgttcctggcaatgacatcgagctgattgaaacgcacgatcaactcgaacagaccgatcagcaggccacccatcatgatggtggcgaaaatgatgttggggtaggtcgccccaagatcgaactcttcctcctcaagcacgccgcccttttccgtcacgttgaatttgcccttggaggggaacagcagggtgacgatggtcacgcgcaccaggaacagcgccatggtggtttcgtacacctcactccagaacgaatagcgccagcccttgttcaccttggcggcggttgcaatggagtggaacatgtgcgggagggcataggccgccacggccagtggcgcggcggcgatgatgttctggcccgcaaacaggaacgccagcggcgaggcaaggaagataacgcgcggaatggcgaagaagaacgacgtcatggccgaaagatagcaaagccgctggcccaacttcaggccgcgcccgagcatcgggttatccacgcggaagatctggatcatgccgcgcgcccagcgcatgcgctggccgatatgggtggtcagtcgctcggtggccagaccactggcaacgggaatgcgcaggtaagcggtggaccagccgcggcgctgcatgcgcagggcggtatgggcatcttccgtcacggtttcaaccgcaaagccgccgatcgattcaatggcctcacgccgcaggatggcgcatgagccgcagaagaaggtggcatcccagaagtcgttgccatcctggatgacgccgtagaacaggttgccttccggcggggtgcggtagcccacggccaggttacgctggaacggatcgggagagtagaagtgatgcggcgtctgcatcagggcgatcttgcggtcagcgaccatccaccccatggcgatctgcaggaacgcgcgtgtcggaatatggtcacaatccaggatgagaatgtaatcgccggaagtccgcttaatggcgtggttgaggttacccgccttggcgtgcgcgctgtcgacacgcccgatatacagggcgccgcaatccttggcgaactgctcgaattcgggccgcacaccgtcatcaaggatatagacattcactttatcgggcggccagtcgatgccgagcgcgcccagcacggtcaggcgcacgatgctcagctgctcatcataggtcgggatgaagatatcgacagtcggccagtcgtcaacattgtcaggcaggggcagcggcgcacgatgaagcggctggattgtctggaaatagctgagaaacagcatgtacagggcatacagctcggccatgagcaggattacgcccagtatgccctgaatccatgtattgaagtcgagcgtttcggtcaggcgccatgtcaggtaacgcagggaaaccagcgcggagagcacctcgagaaaaatctgggtgcgccggctcttgccacgcccgacaacaaaaaagatgacaacacatacagctgccacaattagctgctcattattgttcagcgtaaccgtggtcgcggcaataagtgcacaaagccccagcgctccaactatatagctggccccacgcagtgacagtatcttgttggagatgcggcctagcctactctccgtgggtactggcgactgaacctctgacat

SEQ ID NO: 2 - DNA, 956 bp, Komagataeibacter sucrofermentans
  source 1..956: mol_type = genomic DNA
tatgcctcaccggtcctgtcatcatcgagcacgcgcctgcgtgacttggcgcgcagccagctccatgccccgaacgcggtcagccccgctcctgatagaccggtcaggtaaagaaggaaaggatgataactcagataccggtccagttgcagccacagcggcagcgagcccactttataggttggcgcggtgcggtaactggtaaactgctcggcgttcttgagcaccagatccccctggatggaggacaaatccttggtgttgcgcaggctgagcaccaggtcatggatgcgctgcggtgtatcccccacgaaggcaatgaccgagcggtggctgtcatagggcgactgcgcgccgatcatgaccccggcctcggcaatcggcgcattgaggtgggcggtcacgccgttgaggagacctgcatgatcgtggtcctgaaacaggtaccagatgccctgtagccccatgctctggccaacccgcacgtggccgtccttgatcacgtagggcgagcgtgacagcaggtctgcttgcccattcagccggtcggcggtggagagcaggatgatatcacccttcggggtggtatttttcatctggtctaccgtcatgacatgcacgcctgcggcggggtaccacgttgttgccccgaagaagcccatgaggtcgaggaacgagcctgcggtacctgcatccggggcttgcggcaggatgatcgttgtctcggacagatcggccatgcgggagaacggaaacgcggcctcggcaaaataggacaggttgggcagttcggcgtaatggtagcctcggcggaaatcgagggtggaatctgaatccacgctcatgcggatatcgccaggcgtgcggcggcatgcgccccggtcaatcggtcgggcatcaaaattgaactggagctggttctggccaaacagcagccacggcggcaacgccgtcat

SEQ ID NO: 3 - DNA, 3866 bp, Komagataeibacter sucrofermentans
  source 1..3866: mol_type = genomic DNA
tattgaccgtcaaatgtgtaatgcgccatcaacatgccactggtttctgaccagggaccagcccggctgtagccaccttccatgcccatgcgcaaccgatggttaaactgatagacaatacgcccgcgcatattgccagcaaggccacttgccccattgcccgaataatagtcaggcgggttcgaggccgcgagctgctgcaggctggcacttgtggggtaatagggcgccccgttgctgtgatagtgctggaaccccgcctctccgcgcaggaaccacgtccaccgctgtttatgccccgaccactcaaccggcaccatcgcgccgtaatactgctgtggtgagaagtagccgccctgcccccatgtaaagaagtaactgtcacgcttgtaaccaaaatacatgaggtccaaacccacacgcaaccactgccggtcatgggtctgccataccgtggcggtgccgcctgcaccggcttcgacctcggtattgctctgcacatgcgtgccatcgaggtaggcaaagccgccaccggcatagatattccaccccggcgcggaccattccagcgcgccatggccgaacatgcgcgtcaccccgccccacacccggttcgtgcccggatcgtgcatgcccgcataggacagttcgctatccgtgaccatgcggcggcccccgcttatgcgcaggccgaggttacgggtcagacgcggggcgaattccacgccccccaccacattggtgatggggaagcccagcggagaagaccccacatcggccgagaaccagtgattgacgtagttcaggctcagccccacgccctgcgtatagtaatgatggtatgcccccggcagggctccattgatggaataggtgccgaactgatgggctgaataggaattgttcagcgcatcgcccgtaaacagtagcgtgggcgtgaccgagaaggacagccggtgctcccatgattcaaacggcagcgtgccggttatgggaatggcgaattccgtcagctgccccagccccgcagtacccgtgcggctgcgcacgaagctgttggcgtcgatctgtggcgatatggaatcgcgcagatagacgatctgccggtccatcgcctcggggccatcatcttcggggatgtaatgataggtcgccggcagcgtggctccctgcaggtcgatgtaattgctgtcaatgaagggccagcgataatcgggcaggaagctttcatggccttcatacgcgctttcgccatccagcgtgcgctgggcgcggcgggcgtgttccacatcggcaagctgggcacgcgtgttgcctgccacgcgatcgatatcggagcgcacttcccagctcatcgggccgtcggggtcttcatgcgccagccggtcggcatagctccgcgccagatccattttgctcgcaccgcccgcatcacgcgcggcggcggcgaggccatagatattgcgcggcttgaggcgcagggcaatctggtcttcctccagcgcgcgctggggcatgttgcgtgcctgatatatccggcccatggccagatgcgcctcgactgattcagggtgggcgcgcagcacgggggccatgacctgataggcctgcgtggtctggccgtagcggttgaagttatcggcggtcaggatggcaaggccgatggcgatgtcgtttcttatccgcaactgttccgccgtggcgtagcccggaaagtcgcgagccatcgcatcaaaggtgctgaggcagcgcgtggcgtcgaacgtggcatgcaggcgcaggtacatcccggcataggccagcatctgcgcagccttgggcggctgggtcaggcgctcctcctgcgcgagcacctgctgggcttcacgcgtggcatggcggtcaagcagggcgccagcaatctgcacgccccggtcgcctgtggggtcgggctggctggccagcgccacgagggcggcattatccgcgcgcggcgcgcggttgagcgcctgtatgcggcgggcaagctcgatctggctggcgatgctgttcatgccagcgctccgcccggtttcaggcaggcgcgcgagcaggcgctcggccgtggtcaggtcatgttgccccatggcgtagatgatcccggcctgcaggtcatctggcgtgacggattttgcgtctgtcaggtcattcatcaggctctgcgcctgaaaatggccgcctgcatcatcaagcgcgtgggcaagcttgaggcggacccacgggtctgtgggctcaatggccacggcctggcgcagcagggcaacgcgttcgtcggtatcgcgcgtgcgatcggcgcgggcggaaaggtcggcggcctgtaggtgtgccgccagcgccgggcgcagcggtttgaggcgtacgatgatatcctgcgcttccgccccgcgcccggtctggatcaggatgccgcccagattgaacagcgcatcggcatcactcggcgcccggctcaggatttcgcggtagatgcgctcggcttccgcgtcatgcccctgtctgcgctcgagcatgccttccagcgacagataggtcagcccattgccggagcggtggcccagcagggcaagatccgtgcgggcggcttcgtaatggccgttattgatggcctgcaggatgcgcaccaccagcgggtccatgccacccacgccagattgcagcgccttgatggcagcccgccagtgcggcgctgaatccgggtcagcctgtatggcctgcaaaaaatactgcgtggcctgggcaggctgttgccgggcctgcgccaccagccccaatccgcccagcgcatcggcatcatgggcattgagcgcgagggcgcgatgaaagcgttccgatgccccttccaggttgtggcgggacagcagggcatagccctcctggtgggcggttgcggcgtcgacgccgttctgcgtttcctgcgccttgtgcagcagttcgctcacttccgtatcatcggggtgcaggccaagccattcattatagagcggaatggtagggccagtgatcggctcccacaggagcgcctcgcgccatgcggcaacggccccttccctgatgcccgcaggcacgttggagcgggcaagcgcgcgcaggccgtccatgccctccgggcgcgacgtgacgcgataggtcaggatccggtccagcagcagccgggcatcaagatcgcgcgggttgcgctgcacccaggcggtcagtttggtctgggcttcctggcggccaagaatggtggcccccagcacgcggtaatattccagcgccagatcgggtggcgggtcgccgttcttgaacagggctttgtacttgaacatggcgggcatcatcttgcctgccgccgcaagggcgcgcgcctcggccaggcccccggggtctacggggccagcctgtatctgcgccttgaggtcggcaaccagccctggcaccgagccctggcgctccagccgggccagcgtggccgaggcctgcgccgggttgccctgtgccatctgcaggcggccctgcaggtacagcgcttcagggttattgggctcgagcgaaagcgagcgttctatcgtttcgcgcgctttatcaaggttatgctgccccagccagtaatagccctggttgagcagcagttcgagcacggcggccgcatgcgccatgtgcgcattcatggccgcgcgctgtgcatcctgctcctgcgtgggcgtgaccgtgatggctgtgccatctgtcgccgccgggctgttctgcgtggcctgggcggggtccacctgagcctgcgccatctcgcccgacaggacgacccctgccatcatgccgcagatgaacttcagcgtgctacttgccgcgcgcatgggctggggcgccat

SEQ ID NO: 4 - DNA, 470 bp, Komagataeibacter sucrofermentans
  source 1..470: mol_type = genomic DNA
caggtcgcggcgctgcgggtgcgcatgtacaggatgaccgtctgggccgggaccgagttcaggtcttccgcgtcgatatcacgcgtcacgacataatcaccgaaggcgccgggctgcgacgtgatccagcggccataaagcccttccagcaccggggcaagccatgtgccggcgggttcgcccgcgctgcccacctgcggcaggtcttcatgcacgatgcgcatggcctgttcttccgccagcaggtccagctttacgtagccccagttgatcatggccagcagggcgttcagctcgatctggagctggtggatggtgttgcacagcggcggctggaaacgaccagccataccccggccgacctcgcgcaacaggtcattcctgacctcgatcccggcctgatcatcgatctcccaggacagtgcctgcaggaaaagcgaaaagtccggttttgcgttcaaagttgtcat

SEQ ID NO: 5 - DNA, 2330 bp, Komagataeibacter sucrofermentans
  source 1..2330: mol_type = genomic DNA
cagtcagcagcttcggcttcgcgggtgctgtcgccttcatcgccttcgggggaatcgttttccgcctgcgagatatattcaaagtcgagcttgccatccttgagcgtgatcttggcaaccccgcccttggtcagcttgccaaacagcagttcctcggccagcggcttcttgatgttttcctgaatgacacggcccagggggcgcgcgccatacaggcggtcgtagccacgttcggccagccattcccgcgcggcggacgagatctcgatcatcacgttgcgatcagccaactgggcttcaagctggaagatgaacttctccaccacccggtccaccacatgcggcgacaggttggcgaacggaatgatcgcatcaagccggttgcggaactccggcgtgaacaggcgcttgatcgcatcctcgtcctcgccttcgcgactggtgcggccaaaaccgatggcctccttgctcaggtcggcggcgcccgcgttcgtggtcatgatcagcaccacgttgcggaaatcgaccgtcttgccgttatggtcggtcagccgcccatggtccatcacctgcagcagcacgttatacagatcctgatgcgccttctcgatttcatcaagcagcaggaccgcatgcgggtgctggtcaatggcatcggtcagcaggccaccctggtcaaagcccacatagcccggcggtgcgccgatcagccgcgagatcgaatgccgctccatgtattccgacatgtcgaagcggatcagctcaatgcccagcgttgccgcaagctgcttggccacttccgtcttgcccacgcccgtggggccggagaacaggtagttgccaatcggcttttccgggtcgcgcaggcccgcgcgtgacagcttgatcgcggccgtcagggcctcgatcgccttgtcctgcccgtacaccatgcccttgaggtcacgctcgagcgaacgcagggtttccttgtcgtccgacgagacgctcttgggcgggatgcgggcgatcttcgccacgatgtcttccacatccttcagcgtaacggtcttgcggcggcggttctcgggcaccagcatgcgcgaggcgccaacctcgtcaatcacgtcgatggccttgtcgggcagcttgcggtcgtggatgtacttggcggcaagttccaccgccccacggatcgcatcatcggtgtagcgcaccttgtggtgcttctcgtaattgaccttgaggccacgcaggatcttgatcgcatcctcgaccgaaggctccgccacgtcgatcttctggaaccggcgtacgagtgcacggtctttctcgaagtgctggcggtattccttgtaggtggtcgagcccatgcagcgcagcgtgccggcggcaagggcgggcttgagcaggttggaggcatccatcgccccgcccgaggtggcgcccgcgccaatcacggtatggatctcgtcaatgaacaggatcgagccgggattgttgtcgagttcggtcacgaccgccttcagccgttcctcgaagtcgccacggtagcgcgtgcccgcaagcagcgcgcccatgtcgagcgagtagatggtggcgttgagcagcacttcaggcacgtcgccttcaacgatgcgcttggccagcccttcggcaatggcggtcttgcccacgccggggtcgcctacgtaaagcgggttgttcttggtgcggcggcacaggatctggatcgtgcgctcgatttcagagtcgcggccgatcagcgggtcgaccttgccttcctgcgccttgtcattgaggttggtgcagtaggtggacagcgcatcctggttcttctgcccggtcttgccgcgctcctcggtctcgccgccttcgggcgggctgcccgcaaccgggcggcgcgtggagcggtcgggtgccttggcaatgccgtgggagatgaagttgaccgcatcaagccgcgtcatgtcctgcaactgcaggaagtaaacggcatggctctcgcgctcggcaaacagggctacaagcacgttggccccggtcacctcgtcgcgcccggtggactgcacgtgaatggccgcgcgctgaattacgcgctggaaagcggccgtgggcttggggtcaacggtgcggtcggccgcgaggcctgcgagatccttgtcaagaaaatcggtcaggtcggtgcgcagcttgttcagatcgaccccgcaggcgcggaataccgttacggcatcagggtcatcgatcagcgcgaggaggaggtgttcaagcgttgcgtattcgtgccggcggtcgccagccagtgtcagcgcacggtgaagcgtctgttcaagattacgtgacaacat

SEQ ID NO: 6 - protein, 776 aa, Komagataeibacter sucrofermentans
MLSRNLEQTLHRALTLAGDRRHEYATLEHLLLALIDDPDAVTVFRACGVDLNKLRTDLTDFLDKDLAGLAADRTVDPKPTAAFQRVIQRAAIHVQSTGRDEVTGANVLVALFAERESHAVYFLQLQDMTRLDAVNFISHGIAKAPDRSTRRPVAGSPPEGGETEERGKTGQKNQDALSTYCTNLNDKAQEGKVDPLIGRDSEIERTIQILCRRTKNNPLYVGDPGVGKTAIAEGLAKRIVEGDVPEVLLNATIYSLDMGALLAGTRYRGDFEERLKAVVTELDNNPGSILFIDEIHTVIGAGATSGGAMDASNLLKPALAAGTLRCMGSTTYKEYRQHFEKDRALVRRFQKIDVAEPSVEDAIKILRGLKVNYEKHHKVRYTDDAIRGAVELAAKYIHDRKLPDKAIDVIDEVGASRMLVPENRRRKTVTLKDVEDIVAKIARIPPKSVSSDDKETLRSLERDLKGMVYGQDKAIEALTAAIKLSRAGLRDPEKPIGNYLFSGPTGVGKTEVAKQLAATLGIELIRFDMSEYMERHSISRLIGAPPGYVGFDQGGLLTDAIDQHPHAVLLLDEIEKAHQDLYNVLLQVMDHGRLTDHNGKTVDFRNVVLIMTTNAGAADLSKEAIGFGRTSREGEDEDAIKRLFTPEFRNRLDAIIPFANLSPHVVDRVVEKFIFQLEAQLADRNVMIEISSAAREWLAERGYDRLYGARPLGRVIQENIKKPLAEELLFGKLTKGGVAKITLKDGKLDFEYISQAENDSPEGDEGDSTREAEAAD

SEQ ID NO: 7 - DNA, 503 bp, Komagataeibacter sucrofermentans
  source 1..503: mol_type = genomic DNA
cagtccttttcgatcgtgcattgcagcgggtgctggttctggcgcgcgaggtccatcacctgcgttaccttggtttcggcaacctcgtacgtaaagaccccgcacacgcccacgccacgtttgtgaacgtggagcatgatgtcagtcgcttcctcgcggtttttctggaaaaagcgctcgagcacatgcaccacgaattccatgggcgtgtaatcatcattgagcatcagcaccttgtacatcgccggcttgcgggtctgtggccgggtgcggatgaccacgtcgatcatgccgtcatcattgcccggcggcgagtcctgcccgccgttacggcgcgggggcgtattgcccccatgcccatatgggcgcgggctgtccgcgcagggtcggggcgcggggtggggcagggaaacttgagcaatagaagacatgacaggtaccatattggaactttgccgccggttgaaaggggcgagcgccggggggcagggatttttttgcat

SEQ ID NO: 8 - protein, 167 aa, Komagataeibacter sucrofermentans
MQKNPCPPALAPFNRRQSSNMVPVMSSIAQVSLPHPAPRPCADSPRPYGHGGNTPPRRNGGQDSPPGNDDGMIDVVIRTRPQTRKPAMYKVLMLNDDYTPMEFVVHVLERFFQKNREEATDIMLHVHKRGVGVCGVFTYEVAETKVTQVMDLARQNQHPLQCTIEKD

SEQ ID NO: 9 - DNA, 2277 bp, Escherichia coli
  source 1..2277: mol_type = genomic DNA
atgctcaatcaagaactggaactcagtttaaatatggctttcgccagagcgcgcgagcaccgtcatgagtttatgaccgtcgagcacttgttactggcgctgctcagtaacccatctgcccgggaggcgctggaagcgtgttctgtggatttggttgcgctccgtcaggaactggaagcctttattgaacaaaccacacccgttctgcctgccagtgaagaggagcgcgacacacagccgacgctgagttttcagcgtgtactgcaacgtgcggtcttccatgtccagtcctccggtcgcaatgaggttaccggtgcaaacgttctggtcgctatctttagcgaacaggagtcgcaggcggcatatctgttgcgtaaacatgaagtcagccgtctcgatgtggtgaactttatctctcatggcacgcgtaaagacgagccgacacagtcttctgatcctggcagccagccaaacagcgaagaacaagctggtggggaggaacgtatggagaatttcacgacgaacctgaatcagcttgcgcgcgtgggcggaatcgacccactgattggtcgtgagaaggagctggagcgtgctattcaggttctctgccgtcgccgtaaaaacaacccgctgctggtgggggaatctggtgtcggtaaaaccgcgattgcggaaggtcttgcctggcgaattgttcagggcgatgtgccggaagtgatggctgactgtacgatttactctctcgatatcggttctctgttagcgggcacaaaatatcgcggcgactttgaaaaacgttttaaagcgttgctcaagcagctggagcaggacactaacagcatcctgtttattgatgagatccacaccattatcggtgcgggtgcagcgtctggtggtcaggtcgatgcggctaacctaatcaaaccgttgctctccagcggtaaaattcgtgtaattggttcgacaacctatcaggagttcagcaacattttcgagaaagaccgtgctctggcgcgtcgcttccagaaaattgatattactgaaccgtcgatcgaagaaactgttcaaatcatcaatggcctgaaaccgaagtatgaagcgcaccacgacgtgcgttataccgcaaaagcggtgcgtgcggcggtagagctggcggtgaaatacattaacgatcgtcatctgccggataaagccattgatgttatcgacgaagcgggcgctcgcgcacgcctgatgccggtaagcaaacgcaagaaaaccgttaatgtggcggatattgagtccgtggtggcccgtattgcacgcattccagagaagagtgtttctcagagtgatcgtgataccctgaaaaacctcggcgatcgcttgaaaatgctggtcttcggtcaggataaagccattgaggcgctgactgaagccattaagatggcgcgtgcaggtttaggtcacgaacataaaccggttggttcgttcctgtttgccggccctaccggggtcgggaaaacagaggtgacggtacagctttcgaaagctttgggcattgagcttctgcgctttgatatgtccgagtatatggaacgccataccgtcagccgtcttattggtgcgcctccgggatacgttggttttgatcagggcggtttgctgactgatgcggtcatcaagcatccacatgcggtgctgctgctggacgaaatcgagaaagcgcacccggacgtgttcaatattctgttgcaggtgatggataacggtacgctgaccgataacaacggacgcaaagcagacttccgtaacgtggtgctggtgatgaccaccaacgccggggtacgggaaactgagcgcaaatccattggtcttatccaccaggataacagcaccgatgcgatggaagagatcaagaagatctttacaccggaattccgtaaccgtctcgacaacattatctggtttgatcatctgtcaaccgacgtgatccatcaggtggtggataaattcatcgtcgagttgcaggttcagctggatcagaaaggtgtttctctggaagtgagccaggaagcgcgtaactggctggccgagaaaggttacgaccgggcaatgggcgctcgtccgatggcgcgtgtcatccaggacaacctgaaaaaaccgctcgccaacgaactgctgtttggttcgctggtggacggcggtcaggtcaccgtcgcgctggataaagagaaaaatgagctgacttacggattccagagtgcacaaaagcacaaggcggaagcagcgcattaa

SEQ ID NO: 10 - protein, 758 aa, Escherichia coli
MLNQELELSLNMAFARAREHRHEFMTVEHLLLALLSNPSAREALEACSVDLVALRQELEAFIEQTTPVLPASEEERDTQPTLSFQRVLQRAVFHVQSSGRNEVTGANVLVAIFSEQESQAAYLLRKHEVSRLDVVNFISHGTRKDEPTQSSDPGSQPNSEEQAGGEERMENFTTNLNQLARVGGIDPLIGREKELERAIQVLCRRRKNNPLLVGESGVGKTAIAEGLAWRIVQGDVPEVMADCTIYSLDIGSLLAGTKYRGDFEKRFKALLKQLEQDTNSILFIDEIHTIIGAGAASGGQVDAANLIKPLLSSGKIRVIGSTTYQEFSNIFEKDRALARRFQKIDITEPSIEETVQIINGLKPKYEAHHDVRYTAKAVRAAVELAVKYINDRHLPDKAIDVIDEAGARARLMPVSKRKKTVNVADIESVVARIARIPEKSVSQSDRDTLKNLGDRLKMLVFGQDKAIEALTEAIKMARAGLGHEHKPVGSFLFAGPTGVGKTEVTVQLSKALGIELLRFDMSEYMERHTVSRLIGAPPGYVGFDQGGLLTDAVIKHPHAVLLLDEIEKAHPDVFNILLQVMDNGTLTDNNGRKADFRNVVLVMTTNAGVRETERKSIGLIHQDNSTDAMEEIKKIFTPEFRNRLDNIIWFDHLSTDVIHQVVDKFIVELQVQLDQKGVSLEVSQEARNWLAEKGYDRAMGARPMARVIQDNLKKPLANELLFGSLVDGGQVTVALDKEKNELTYGFQSAQKHKAEAAH

SEQ ID NO: 11 - DNA, 321 bp, Escherichia coli
  source 1..321: mol_type = genomic DNA
atgggtaaaacgaacgactggctggactttgatcaactggcggaagaaaaagttcgcgacgcgctaaaaccgccatctatgtataaagtgatattagtcaatgatgattacactccgatggagtttgttattgacgtgttacaaaaattcttttcttatgatgtagaacgtgcaacgcaattgatgctcgctgttcactaccaggggaaggccatttgcggagtctttaccgccgaggttgcagaaaccaaagtggcgatggtgaacaagtacgcgagggagaatgagcatccattgctgtgtacgctagaaaaagcctga

SEQ ID NO: 12 - protein, 106 aa, Escherichia coli
MGKTNDWLDFDQLAEEKVRDALKPPSMYKVILVNDDYTPMEFVIDVLQKFFSYDVERATQLMLAVHYQGKAICGVFTAEVAETKVAMVNKYARENEHPLLCTLEKA

SEQ ID NO: 13 - DNA, 4705 bp, synthetic construct
  source 1..4705: mol_type = other DNA
gacgaaagggcctcgtgatacgcctatttttataggttaatgtcatgataataatggtttcttagacgtcaggtggcacttttcggggaaatgtgcgcggaacccctatttgtttatttttctaaatacattcaaatatgtatccgctcatgagacaataaccctgataaatgcttcaataatattgaaaaaggaagagtatgagtattcaacatttccgtgtcgcccttattcccttttttgcggcattttgccttcctgtttttgctcacccagaaacgctggtgaaagtaaaagatgctgaagatcagttgggtgcacgagtgggttacatcgaactggatctcaacagcggtaagatccttgagagttttcgccccgaagaacgttttccaatgatgagcacttttaaagttctgctatgtggcgcggtattatcccgtattgacgccgggcaagagcaactcggtcgccgcatacactattctcagaatgacttggttgagtactcaccagtcacagaaaagcatcttacggatggcatgacagtaagagaattatgcagtgctgccataaccatgagtgataacactgcggccaacttacttctgacaacgatcggaggaccgaaggagctaaccgcttttttgcacaacatgggggatcatgtaactcgccttgatcgttgggaaccggagctgaatgaagccataccaaacgacgagcgtgacaccacgatgcctgtagcaatggcaacaacgttgcgcaaactattaactggcgaactacttactctagcttcccggcaacaattaatagactggatggaggcggataaagttgcaggaccacttctgcgctcggcccttccggctggctggtttattgctgataaatctggagccggtgagcgtgggtctcgcggtatcattgcagcactggggccagatggtaagccctcccgtatcgtagttatctacacgacggggagtcaggcaactatggatgaacgaaatagacagatcgctgagataggtgcctcactgattaagcattggtaactgtcagaccaagtttactcatatatactttagattgatttaaaacttcatttttaatttaaaaggatctaggtgaagatcctttttgataatctcatgaccaaaatcccttaacgtgagttttcgttccactgagcgtcagaccccgtagaaaagatcaaaggatcttcttgagatcctttttttctgcgcgtaatctgctgcttgcaaacaaaaaaaccaccgctaccagcggtggtttgtttgccggatcaagagctaccaactctttttccgaaggtaactggcttcagcagagcgcagataccaaatactgttcttctagtgtagccgtagttaggccaccacttcaagaactctgtagcaccgcctacatacctcgctctgctaatcctgttaccagtggctgctgccagtggcgataagtcgtgtcttaccgggttggactcaagacgatagttaccggataaggcgcagcggtcgggctgaacggggggttcgtgcacacagcccagcttggagcgaacgacctacaccgaactgagatacctacagcgtgagctatgagaaagcgccacgcttcccgaagggagaaaggcggacaggtatccggtaagcggcagggtcggaacaggagagcgcacgagggagcttccagggggaaacgcctggtatctttatagtcctgtcgggtttcgccacctctgacttgagcgtcgatttttgtgatgctcgtcaggggggcggagcctatggaaaaacgccagcaacgcggcctttttacggttcctggccttttgctggccttttgctcacatgttctttcctgcgttatcccctgattctgtggataaccgtattaccgcctttgagtgagctgataccgctcgccgcagccgaacgaccgagcgcagcgagtcagtgagcgaggaagcggaagagcgcccaatacgcaaaccgcctctccccgcgcgttggccgattcattaatgcagctggcacgacaggtttcccgactggaaagcgggcagtgagcgcaacgcaattaatgtgagttagctcactcattaggcaccccaggctttacactttatgcttccggctcgtatgttgtgtggaattgtgagcggataacaatttcacacaggaaacagctatgaccatgattacgccaagcttgcatgcctgcaggtcgactctagaggatccccgggtaccgagctcgaattcactggccgtcgttttacaacgtcgtgactgggaaaaccctggcgggccaagcttggagggctccatcgaggcggcgtgaaccgaaaccggcatttcctgattaaatgcaacctgccccgtgcgcacggccttgaaagcgaggtaaagcgtcatcagcttggtcaggctggcggggtagcgacgcaggtccgaatcctgctgcgacagcacggccccggtgcgggcatcgaccacgatggagctgacctgccccacatattgcgcccttgccgcctgcatgcccccaaggccgacacacagccccacggttacagtgaccttgaggcgggaaaaacgggtagcggataaacggctcatgggatggcgaaacctgcgcgtgcaatcatcatcatacggcttcgggcgcacggggttacccggcacccctccatccattcacgggttgcttggctgcaaccattctaaaagaaaggttttctattcgtccagagcgtatttatatccttgccattccataaacgcgggcggcagcggatcagggcacggcaaaatcctgtatatcgtgcgaaaaaggatggatataccgaaaaaatcgctataatgaccccgaagcagggttatgcagcggaaaaggacaaaagtcaaattacgccccgccctgccactcatcgcagtactgttgtaattcattaagcattctgccgacatggaagccatcacaaacggcatgatgaacctgaatcgccagcggcatcagcaccttgtcgccttgcgtataatatttgcccatggtgaaaacgggggcgaagaagttgtccatattggccacgtttaaatcaaaactggtgaaactcacccagggattggctgagacgaaaaacatattctcaataaaccctttagggaaataggccaggttttcaccgtaacacgccacatcttgcgaatatatgtgtagaaactgccggaaatcgtcgtggtattcactccagagcgatgaaaacgtttcagtttgctcatggaaaacggtgtaacaagggtgaacactatcccatatcaccagctcaccgtctttcattgccatacgaaattccggatgagcattcatcaggcgggcaagaatgtgaataaaggccggataaaacttgtgcttatttttctttacggtctttaaaaaggccgtaatatccagctgaacggtctggttataggtacattgagcaactgactgaaatgcctcaaaatgttctttacgatgccattgggatatatcaacggtggtatatccagtgatttttttctccattttagcttccttagctcctgaaaatctcgataactcaaaaaatacgcccggtagtgatcttatttcattatggtgaaagttggaacctcttacgtgccgatcaacgtctcattttcgccaatttaaatcgtaattattggggacccctggattctcaccaataaaaaacgcccggcggcaaccgagcgttctgaacaaatccagatggagttctgaggtcattactggatctatcaacaggagtccaagctgcagcggcccaaaaaaatccctgccccccggcgctcgcccctttcaaccggcggcaaagttccaatatggtacctgtcatgtcttctattgctcaagtttccctgccccaccccgcgccccgaccctgcgcggacagcccgcgcccatatgggcatgggggcaatacgcccccgcgccgtaacggcgggcaggactcgccgccgggcaatgatgacggcatgatcgacgtggtcatccgcacccggccacagacccgcaagccggcgatgtacaaggtgctgatgctcaatgatgattacacgcccatggaattcgtggtgcatgtgctcgagcgctttttccagaaaaaccgcgaggaagcgactgacatcatgctccacgttcacaaacgtggcgtgggcgtgtgcggggtctttacgtacgaggttgccgaaaccaaggtaacgcaggtgatggacctcgcgcgccagaaccagcacccgctgcaatgcacgatcgaaaaggattacccaacttaatcgccttgcagcacatccccctttcgccagctggcgtaatagcgaagaggcccgcaccgatcgcccttcccaacagttgcgcagcctgaatggcgaatggcgcctgatgcggtattttctccttacgcatctgtgcggtatttcacaccgcatatggtgcactctcagtacaatctgctctgatgccgcatagttaagccagccccgacacccgccaacacccgctgacgcgccctgacgggcttgtctgctcccggcatccgcttacagacaagctgtgaccgtctccgggagctgcatgtgtcagaggttttcaccgtcatcaccgaaacgcgcga